European Patent Application EP 4 342 530 A1, published March 27, 2024. Title: COMPOUNDS. Applicant: Insusense ApS. Application EP, filed September 2, 2022. The sequence listing filed with the application follows.

SEQUENCE LISTING (4 sequences)

SEQ ID NO: 1 - protein, 831 aa, Homo sapiens [sequence omitted]

SEQ ID NO: 2 - protein, 830 aa, Homo sapiens
MERPWGAADGLSRWPHGLGLLLLLQLLPPSTLSQDRLDAPPPPAAPLPRWSGPIGVSWGLRAAAAGGAFPRGGRWRRSAPGEDEECGRVRDFVAKLANNTHQHVFDDLRGSVSLSWVGDSTGVILVLTTFHVPLVIMTFGQSKLYRSEDYGKNFKDITDLINNTFIRTEFGMAIGPENSGKVVLTAEVSGGSRGGRIFRSSDFAKNFVQTDLPFHPLTQMMYSPQNSDYLLALSTENGLWVSKNFGGKWEEIHKAVCLAKWGSDNTIFFTTYANGSCTDLGALELWRTSDLGKSFKTIGVKIYSFGLGGRFLFASVMADKDTTRRIHVSTDQGDTWSMAQLPSVGQEQFYSILAANDDMVFMHVDEPGDTGFGTIFTSDDRGIVYSKSLDRHLYTTTGGETDFTNVTSLRGVYITSVLSEDNSIQTMITFDQGGRWTHLRKPENSECDATAKNKNECSLHIHASYSISQKLNVPMAPLSEPNAVGIVIAHGSVGDAISVMVPDVYISDDGGYSWTKMLEGPHYYTILDSGGIIVAIEHSSRPINVIKFSTDEGQCWQTYTFTRDPIYFTGLASEPGARSMNISIWGFTESFLTSQWVSYTIDFKDILERNCEEKDYTIWLAHSTDPEDYEDGCILGYKEQFLRLRKSSVCQNGRDYVVTKQPSICLCSLEDFLCDFGYYRPENDSKCVEQPELKGHDLEFCLYGREEHLTTNGYRKIPGDKCQGGVNPVREVKDLKKKCTSNFLSPEKQNSKSNSVPIILAIVGLMLVTVVAGVLIVKKYVCGGRFLVHRYSVLQQHAEANGVDGVDALDTASHTNKSGYHDDSDEDLLE

SEQ ID NO: 3 - protein, 694 aa, Homo sapiens
MTFGQSKLYRSEDYGKNFKDITDLINNTFIRTEFGMAIGPENSGKVVLTAEVSGGSRGGRIFRSSDFAKNFVQTDLPFHPLTQMMYSPQNSDYLLALSTENGLWVSKNFGGKWEEIHKAVCLAKWGSDNTIFFTTYANGSCTDLGALELWRTSDLGKSFKTIGVKIYSFGLGGRFLFASVMADKDTTRRIHVSTDQGDTWSMAQLPSVGQEQFYSILAANDDMVFMHVDEPGDTGFGTIFTSDDRGIVYSKSLDRHLYTTTGGETDFTNVTSLRGVYITSVLSEDNSIQTMITFDQGGRWTHLRKPENSECDATAKNKNECSLHIHASYSISQKLNVPMAPLSEPNAVGIVIAHGSVGDAISVMVPDVYISDDGGYSWTKMLEGPHYYTILDSGGIIVAIEHSSRPINVIKFSTDEGQCWQTYTFTRDPIYFTGLASEPGARSMNISIWGFTESFLTSQWVSYTIDFKDILERNCEEKDYTIWLAHSTDPEDYEDGCILGYKEQFLRLRKSSVCQNGRDYVVTKQPSICLCSLEDFLCDFGYYRPENDSKCVEQPELKGHDLEFCLYGREEHLTTNGYRKIPGDKCQGGVNPVREVKDLKKKCTSNFLSPEKQNSKSNSVPIILAIVGLMLVTVVAGVLIVKKYVCGGRFLVHRYSVLQQHAEANGVDGVDALDTASHTNKSGYHDDSDEDLLE

SEQ ID NO: 4 - protein, 825 aa, Mus musculus
MERPRGAADGLLRWPLGLLLLLQLLPPAAVGQDRLDAPPPPAPPLLRWAGPVGVSWGLRAAAPGGPVPRAGRWRRGAPAEDQDCGRLPDFIAKLTNNTHQHVFDDLSGSVSLSWVGDSTGVILVLTTFQVPLVIVSFGQSKLYRSEDYGKNFKDITNLINNTFIRTEFGMAIGPENSGKVILTAEVSGGSRGGRVFRSSDFAKNFVQTDLPFHPLTQMMYSPQNSDYLLALSTENGLWVSKNFGEKWEEIHKAVCLAKWGPNNIIFFTTHVNGSCKADLGALELWRTSDLGKTFKTIGVKIYSFGLGGRFLFASVMADKDTTRRIHVSTDQGDTWSMAQLPSVGQEQFYSILAANEDMVFMHVDEPGDTGFGTIFTSDDRGIVYSKSLDRHLYTTTGGETDFTNVTSLRGVYITSTLSEDNSIQSMITFDQGGRWEHLRKPENSKCDATAKNKNECSLHIHASYSISQKLNVPMAPLSEPNAVGIVIAHGSVGDAISVMVPDVYISDDGGYSWAKMLEGPHYYTILDSGGIIVAIEHSNRPINVIKFSTDEGQCWQSYVFTQEPIYFTGLASEPGARSMNISIWGFTESFITRQWVSYTVDFKDILERNCEEDDYTTWLAHSTDPGDYKDGCILGYKEQFLRLRKSSVCQNGRDYVVAKQPSVCPCSLEDFLCDFGYFRPENASECVEQPELKGHELEFCLYGKEEHLTTNGYRKIPGDKCQGGMNPAREVKDLKKKCTSNFLNPTKQNSKSNSVPIILAIVGLMLVTVVAGVLIVKKYVCGGRFLVHRYSVLQQHAEADGVEALDSTSHAKSGYHDDSDEDLLE